European Patent Application EP 4 260 873 A1, published October 18, 2023. Title: COMBINATION DRUG FOR TREATING KIDNEY CANCER AND POTENTIATOR FOR THERAPEUTIC EFFECTS OF TYROSINE KINASE INHIBITOR. Applicant: Saitama Medical University. The sequence listing filed with the application follows.

SEQUENCE LISTING (36 sequences)

SEQ ID NO: 1 - DNA, 21 bp, Artificial Sequence
  target sequence
ggagggtacgtaacctcaatg

SEQ ID NO: 2 - RNA, 21 nt, Artificial Sequence
  siDPP4 #1, Sense
ggaggguacguaaccucaaug

SEQ ID NO: 3 - RNA, 21 nt, Artificial Sequence
  siDPP4 #1, Antisense
uugagguuacguacccuccau

SEQ ID NO: 4 - DNA, 21 bp, Artificial Sequence
  target sequence
cagtcgcaaaacttacactct

SEQ ID NO: 5 - RNA, 21 nt, Artificial Sequence
  siDPP4 #2, Sense
cagucgcaaaacuuacacucu

SEQ ID NO: 6 - RNA, 21 nt, Artificial Sequence
  siDPP4 #2, Antisense
aguguaaguuuugcgacuguc

SEQ ID NO: 7 - RNA, 21 nt, Artificial Sequence
  siControl, Sense
guaccgcacgucauucguauc

SEQ ID NO: 8 - RNA, 21 nt, Artificial Sequence
  siControl, Antisense
uacgaaugacgugcgguacgu

SEQ ID NO: 9 - DNA, 21 bp, Artificial Sequence
  primer
ccaaacggcacttttttagca

SEQ ID NO: 10 - DNA, 28 bp, Artificial Sequence
  primer
gagtattcaataagtgggacttctgtgt

SEQ ID NO: 11 - DNA, 18 bp, Artificial Sequence
  primer
gtgatggcacccgctatg

SEQ ID NO: 12 - DNA, 20 bp, Artificial Sequence
  primer
actgtcttcgtctgggatgg

SEQ ID NO: 13 - DNA, 21 bp, Artificial Sequence
  primer
cagagtacaaacgccaaacca

SEQ ID NO: 14 - DNA, 20 bp, Artificial Sequence
  primer
aaatcacgatgagggtcagc

SEQ ID NO: 15 - DNA, 20 bp, Artificial Sequence
  primer
ttcagccaaacgaccatctg

SEQ ID NO: 16 - DNA, 20 bp, Artificial Sequence
  primer
cacgagggtttctgctttgc

SEQ ID NO: 17 - DNA, 22 bp, Artificial Sequence
  primer
gcatgacggacaagtacaggct

SEQ ID NO: 18 - DNA, 21 bp, Artificial Sequence
  primer
aaagtaccagtttgccacggc

SEQ ID NO: 19 - DNA, 21 bp, Artificial Sequence
  primer
cgcaagacaggcttttcagat

SEQ ID NO: 20 - DNA, 18 bp, Artificial Sequence
  primer
ccctctcggaagcatcca

SEQ ID NO: 21 - DNA, 20 bp, Artificial Sequence
  primer
aggccctcacagtgtcttct

SEQ ID NO: 22 - DNA, 20 bp, Artificial Sequence
  primer
acatcttgaatcccccaaag

SEQ ID NO: 23 - DNA, 20 bp, Artificial Sequence
  primer
tggatcaactgctacaacgc

SEQ ID NO: 24 - DNA, 20 bp, Artificial Sequence
  primer
cacttctgtgtattcggcca

SEQ ID NO: 25 - DNA, 23 bp, Artificial Sequence
  primer
agacagccactcacctcttcaga

SEQ ID NO: 26 - DNA, 21 bp, Artificial Sequence
  primer
cagccatctttggaaggttca

SEQ ID NO: 27 - DNA, 19 bp, Artificial Sequence
  primer
ccacgctgctgaacatgct

SEQ ID NO: 28 - DNA, 20 bp, Artificial Sequence
  primer
gatgctgccattgtcgaaca

SEQ ID NO: 29 - DNA, 24 bp, Artificial Sequence
  primer
ctaatgtgttggccagctgctacc

SEQ ID NO: 30 - DNA, 24 bp, Artificial Sequence
  primer
gtccgatggggcattaccacatga

SEQ ID NO: 31 - DNA, 24 bp, Artificial Sequence
  primer
cctcttcaaggggactaactacaa

SEQ ID NO: 32 - DNA, 24 bp, Artificial Sequence
  primer
ctatcattgcaagattgctctctc

SEQ ID NO: 33 - DNA, 46 bp, Artificial Sequence
  primer
ctctagaaagactggtgacacagaggtcaaggtgggggaggcatga

SEQ ID NO: 34 - DNA, 54 bp, Artificial Sequence
  primer
catggagatctttctgaccactgtgtctccagttccaccccctccgtactgcgc

SEQ ID NO: 35 - DNA, 46 bp, Artificial Sequence
  primer
ctctagaaagaccaacatcacagcaacataggtgcaacatgcatga

SEQ ID NO: 36 - DNA, 54 bp, Artificial Sequence
  primer
cgcgtcatgcatgttgcacctatgttgctgtgatgttggtctttctagaggtac